European Patent Application EP 4 471 158 A1, published December 4, 2024. Title: mRNA and its template for protein expression. Applicant: SK bioscience Co., Ltd. Application KR. The sequence listing filed with the application follows.

SEQUENCE LISTING (98 sequences)

SEQ ID NO: 1 - DNA, 111 bp, synthetic construct
  source 1..111: mol_type = other DNA; note = alpha-globin
gctggagcctcggtggccatgcttcttgccccttgggcctccccccagcccctcctccccttcctgcacccgtacccccgtggtctttgaataaagtctgagtgggcggca

SEQ ID NO: 2 - DNA, 56 bp, synthetic construct
  source 1..56: mol_type = other DNA
agaaataagagagaaaagaagagtaagaagaaatataagaccccggcgccgccacc

SEQ ID NO: 3 - DNA, 54 bp, synthetic construct
  source 1..54: mol_type = other DNA; note = Muscle_ASXL3
agcaccccgtggaatcccccacgtcatcatcagaaccatcaatgagatgcaaac

SEQ ID NO: 4 - DNA, 36 bp, synthetic construct
  source 1..36: mol_type = other DNA; note = Muscle_CEP152
agtcgcggtaacagcctccgtggcctccggaggacc

SEQ ID NO: 5 - DNA, 93 bp, synthetic construct
  source 1..93: mol_type = other DNA; note = Muscle_FSIP2
agattcctggtcaggtccggacagagggacaacggggtgctagagaaggagagcggggcgggtgaggaaggggctgagggggctgtgccggcc

SEQ ID NO: 6 - DNA, 29 bp, synthetic construct
  source 1..29: mol_type = other DNA; note = Muscle_PPRC1
agagcagcgctgggtgttcaggggccaag

SEQ ID NO: 7 - DNA, 41 bp, synthetic construct
  source 1..41: mol_type = other DNA; note = Muscle_SAP18
agtaaagtgtcgagcttctcctcgcgagagacttagtgctc

SEQ ID NO: 8 - DNA, 72 bp, synthetic construct
  source 1..72: mol_type = other DNA; note = Muscle_UBE2G2
agtccccggtgtcggggcaggaggcacgcgcgcggctgaggcgaggtcgctcggcgcagctgttgcggggcc

SEQ ID NO: 9 - DNA, 88 bp, synthetic construct
  source 1..88: mol_type = other DNA; note = Muscle_ASB1
agcggcgccggaagtggtcgcgggtcgttctgcttcctgcccgaggggcgtgcgcgggtcaggggcggccgcggaggcggaagcatcc

SEQ ID NO: 10 - DNA, 59 bp, synthetic construct
  source 1..59: mol_type = other DNA; note = Muscle_ITGB1BP2
agattcggcagccagactccttgaaataccctttcagtaatcattcaaccaacgcttcc

SEQ ID NO: 11 - DNA, 76 bp, synthetic construct
  source 1..76: mol_type = other DNA; note = Muscle_S100A1
agccacatttgcaaccttggccatctgtccagaacctgctcccacctcaggcccaggccaaccgtgcactgctgca

SEQ ID NO: 12 - DNA, 60 bp, synthetic construct
  source 1..60: mol_type = other DNA; note = Muscle_CHEK2
agactctgctggctgaggctgcggagagtgtgcggctccaggtgggctcacgcggtcgtg

SEQ ID NO: 13 - DNA, 62 bp, synthetic construct
  source 1..62: mol_type = other DNA; note = Muscle_TUBB3
agctcagcagccagcccggcccgcccgcgcccgtccgcagccgcccgccagacgcgcccagt

SEQ ID NO: 14 - DNA, 38 bp, synthetic construct
  source 1..38: mol_type = other DNA; note = Spleen_DAB1
agcgggatctgtgtgaagtggactaaggattaagtagg

SEQ ID NO: 15 - DNA, 48 bp, synthetic construct
  source 1..48: mol_type = other DNA; note = Spleen_EVC2
aggactcggcggcacccgccgctttgaggtagcgggtcccgacaggcg

SEQ ID NO: 16 - DNA, 56 bp, synthetic construct
  source 1..56: mol_type = other DNA; note = Spleen_PRR9
agtccacagcctttgttgagtcttgttgaagatcaggctctgcaaatcaccctagg

SEQ ID NO: 17 - DNA, 77 bp, synthetic construct
  source 1..77: mol_type = other DNA; note = Spleen_KDM5D
agactgcagggcccggaggtcaagatggtggctgtaaaactaggatccctgacgattgcttagcattaaggcccgac

SEQ ID NO: 18 - DNA, 79 bp, synthetic construct
  source 1..79: mol_type = other DNA; note = Spleen_MITD1
agacatgaccacttcccggaagcgcagcagacccgctcaacttcatcctgggttgaggcggaggagaacttccagaatt

SEQ ID NO: 19 - DNA, 29 bp, synthetic construct
  source 1..29: mol_type = other DNA; note = Spleen_ZNF292
aggcgtacgcgacggagcggggtgtgaag

SEQ ID NO: 20 - DNA, 35 bp, synthetic construct
  source 1..35: mol_type = other DNA; note = Spleen_CDA
agcccgctgctctgctgcctgcccggggtaccaac

SEQ ID NO: 21 - DNA, 72 bp, synthetic construct
  source 1..72: mol_type = other DNA; note = Spleen_PLEK
agatgcagaggaggcccagctgctgagaggagttgcctgagagtgacctttgcatctgcctgtccagccagc

SEQ ID NO: 22 - DNA, 85 bp, synthetic construct
  source 1..85: mol_type = other DNA; note = Spleen_LDB3
agattcttaggagcctctcaagagctccacgcagcccggctgggcagcaagggacagaacagaggcggccgctgacagcaccagc

SEQ ID NO: 23 - DNA, 37 bp, synthetic construct
  source 1..37: mol_type = other DNA; note = Spleen_POSTN
agctcttcggggactaactgcaacggagagactcaag

SEQ ID NO: 24 - DNA, 41 bp, synthetic construct
  source 1..41: mol_type = other DNA; note = Lymphoid_AKIP1
agcgttgcgcgcatgcgccttgacgagtgagccggggagcc

SEQ ID NO: 25 - DNA, 61 bp, synthetic construct
  source 1..61: mol_type = other DNA; note = Lymphoid_CHD6
agctgtttgtattttggctgctgcaggagccattttagaaataaatatcttccttcaatag

SEQ ID NO: 26 - DNA, 90 bp, synthetic construct
  source 1..90: mol_type = other DNA; note = Lymphoid_GRIN2D
agggacgccgggttccggtcctggcccccccgccatccccccaacagaacagggtcatgaaaagaggccgcccggcggggcccgcaggcg

SEQ ID NO: 27 - DNA, 63 bp, synthetic construct
  source 1..63: mol_type = other DNA; note = Lymphoid_CASP2
agcggcccccggtttgtttgggctgtgggcggtgcgcagcggagagcccgggaaaagcgggaa

SEQ ID NO: 28 - DNA, 64 bp, synthetic construct
  source 1..64: mol_type = other DNA; note = Lymphoid_CYTH4
aggaacagcagctgggtcggcaagcgacaggagcacgggtcatcttttccccagaggcgtcgga

SEQ ID NO: 29 - DNA, 58 bp, synthetic construct
  source 1..58: mol_type = other DNA; note = Lymphoid_TNFAIP8
aggctcgtccgagtacatgtgagcggtaatcgcccctgcagctggttatcctgacatt

SEQ ID NO: 30 - DNA, 77 bp, synthetic construct
  source 1..77: mol_type = other DNA; note = Lymphoid_CAMK2B
aggtgcccgcgagcgggagccggagtcgccgccgcccgagcgcagccgagcgcacgccgagcccgtccgccgccgcc

SEQ ID NO: 31 - DNA, 63 bp, synthetic construct
  source 1..63: mol_type = other DNA; note = Lymphoid_HMGCS2
agatctctttcaaggtttctgctgggtttctgaactgctgggtttctgcttgctcctctggag

SEQ ID NO: 32 - DNA, 78 bp, synthetic construct
  source 1..78: mol_type = other DNA; note = Lymphoid_PYGM
agactccttggctggaggcagtgctgaggccgccgtcccctctaccatcagtccagtccggcccgccctcctgcagcc

SEQ ID NO: 33 - DNA, 101 bp, synthetic construct
  source 1..101: mol_type = other DNA; note = Bone Marrow_ZNF33A
agcgtccgccggctacgtctgcgtttccgcctttccttttgtttttctcaggttttgcgtgggaggcggtcccgggatttcaagggtctacgcgcttttct

SEQ ID NO: 34 - DNA, 98 bp, synthetic construct
  source 1..98: mol_type = other DNA; note = Bone Marrow_CCNDBP1
agcttgacgctgtggcccggaagtggagcggctgtcgcagtgcggctccggcagtggcagcggaggcctgtgtttgcggccttcggcaagcgactgag

SEQ ID NO: 35 - DNA, 84 bp, synthetic construct
  source 1..84: mol_type = other DNA; note = Bone Marrow_FECH
agacccggctcggccactgctgggcggacacctgggcgcgccgccgcgggaggagcccggactcgggccgaggctgcccaggca

SEQ ID NO: 36 - DNA, 79 bp, synthetic construct
  source 1..79: mol_type = other DNA; note = Bone Marrow_USP15
aggtgggacgccattcccataatgctctggggcgtgccgccgccgtcgctgccacctcccctaccgctagtggaagaag

SEQ ID NO: 37 - DNA, 87 bp, synthetic construct
  source 1..87: mol_type = other DNA; note = Bone Marrow_ATP1A2
agccgactgtcccagacgggctggtgtgggcttgggatcctcctggtgacctctcccgctaaggtccctcagccactctgccccaag

SEQ ID NO: 38 - DNA, 65 bp, synthetic construct
  source 1..65: mol_type = other DNA; note = Bone Marrow_MT3
agaagccgcgcgtccagttgcttggagaagcccgttcaccgcctccagctgctgctctcctcgac

SEQ ID NO: 39 - DNA, 48 bp, synthetic construct
  source 1..48: mol_type = other DNA; note = Bone Marrow_PKP2
aggcgagtccagaggcaggcgagcagctcggtcgcccccaccggcccc

SEQ ID NO: 40 - DNA, 66 bp, synthetic construct
  source 1..66: mol_type = other DNA; note = High-RPKM_ACTB
agcccgcgagcacagagcctcgcctttgccgatccgccgcccgtccacacccgccgccagctcacc

SEQ ID NO: 41 - DNA, 55 bp, synthetic construct
  source 1..55: mol_type = other DNA; note = High-RPKM_ACTG1
aggggtatccccccgaccgcccgaagctggggagccgaccttcaaaaaagtcgca

SEQ ID NO: 42 - DNA, 53 bp, synthetic construct
  source 1..53: mol_type = other DNA; note = High-RPKM_HBB
agtacatttgcttctgacacaactgtgttcactagcaacctcaaacagacacc

SEQ ID NO: 43 - DNA, 64 bp, synthetic construct
  source 1..64: mol_type = other DNA; note = High-RPKM_RPL19
aggcagataatgggaggagccgggcccgagcgagctctttcctttcgctgctgcggccgcagcc

SEQ ID NO: 44 - DNA, 76 bp, synthetic construct
  source 1..76: mol_type = other DNA; note = High-RPKM_RPLP2
agccttttcctccctgtcgccaccgaggtcgcacgcgtgagacttctccgccgcctccgccgcagacgccgccgcg

SEQ ID NO: 45 - DNA, 47 bp, synthetic construct
  source 1..47: mol_type = other DNA; note = High-RPKM_RPS18
agctctcttccacaggaggcctacacgccgccgcttgtgctgcagcc

SEQ ID NO: 46 - DNA, 45 bp, synthetic construct
  source 1..45: mol_type = other DNA; note = High-RPKM_S100A9
agaaacactctgtgtggctcctcggctttgacagagtgcaagacg

SEQ ID NO: 47 - DNA, 53 bp, synthetic construct
  source 1..53: mol_type = other DNA; note = alpha-globin
agaataaactagtattcttctggtccccacagactcagagagaacccgccacc

SEQ ID NO: 48 - DNA, 295 bp, synthetic construct
  source 1..295: mol_type = other DNA; note = AES and mtRNR
ctcgagctggtactgcatgcacgcaatgctagctgcccctttcccgtcctgggtaccccgagtctcccccgacctcgggtcccaggtatgctcccacctccacctgccccactcaccacctctgctagttccagacacctcccaagcacgcagcaatgcagctcaaaacgcttagcctagccacacccccacgggaaacagcagtgattaacctttagcaataaacgaaagtttaactaagctatactaaccccagggttggtcaatttcgtgccagccacaccctggagctagc

SEQ ID NO: 49 - DNA, 311 bp, synthetic construct
  source 1..311: mol_type = other DNA; note = Muscle_CEP152
ttatggtacagtatttaagaagaatcattaatatattaacaaaaatggaagggaagacctcatactgaaaaaaattgtgagccctgcctcttttgagatgttttaataacatctgttatataagtaaagcattcttctaaaattgcttgagatatttatgttgccttaatattccaaaggcctgatggtgtatgtataatctgcttttgtgtggtgcttatttttggtttctaaaccatctatttttatacttataaattgactcactctgcagtgttaacttatttaaataaacttgcatatggtctgta

SEQ ID NO: 50 - DNA, 82 bp, synthetic construct
  source 1..82: mol_type = other DNA; note = Muscle_DNAH12
attggacaaatttataaaacatccaaaagtttaaaaaaaaaaaaacctgtcctacttaaaatatatacattataaaaccaag

SEQ ID NO: 51 - DNA, 169 bp, synthetic construct
  source 1..169: mol_type = other DNA; note = Muscle_HUS1B
aaattcagccagcttagattttttttttaaggttttgatcttttcaaaactaaaacagaccctgagttaattgggttgaaaatttggaccttcactgacttatgcagggcgtatattttgttgagcccttcctcctttgcaaaatttatattaaagcattggtaaaaca

SEQ ID NO: 52 - DNA, 134 bp, synthetic construct
  source 1..134: mol_type = other DNA; note = Muscle_ATXN7L2
cgagaaagtgcctgcccactgcaacggagccgccagcacctcctcccctccagatccgggccccaggctgctgccgctttttataactttatattatttttttttaagaaaaaaagctctttaaaatacctcaa

SEQ ID NO: 53 - DNA, 106 bp, synthetic construct
  source 1..106: mol_type = other DNA; note = Muscle_ASB1
actccaagtgctgcggttgattccagtgagggagaaagtgatctgcagggaggtggacaccgagccctgagtgctgtgctgctgctggtctcctgatggctgttgc

SEQ ID NO: 54 - DNA, 174 bp, synthetic construct
  source 1..174: mol_type = other DNA; note = Muscle_GPT
gcaccccagctggggccaggctgggtcgccctggactgtgtgctcaggagccctgggaggctctggagcccactgtacttgctcttgatgcctggcggggtggggtggggggggtgctgggcccctgcctctctgcaggtccctaataaagctgtgtggcagtctgactccagg

SEQ ID NO: 55 - DNA, 179 bp, synthetic construct
  source 1..179: mol_type = other DNA; note = Muscle_ITGB1BP2
tgacaccagacagttgatgtctagataggacctcaatgattcccttagaatcttagataccaggatattgttggccatgtggcatcattgagcagcaggaggctgaaggaggggagaacaaaattgtccaaaccatgctgtttttttcccttaaataaatcttgtattcttcagtttca

SEQ ID NO: 56 - DNA, 154 bp, synthetic construct
  source 1..154: mol_type = other DNA; note = Muscle_CHEK2
actccgtggtttgaacacgaaagaaatgtaccttctttcactctgtcatctttcttttctttgagtctgtttttttatagtttgtattttaattatgggaataattgctttttcacagtcactgatgtacaattaaaaacctgatggaacctgg

SEQ ID NO: 57 - DNA, 307 bp, synthetic construct
  source 1..307: mol_type = other DNA; note = Muscle_SPRR2G
catcactagaattcatcaggaccatgaaacaacaagatccagtggctcttcttactcccaggactccatcatcttcccttcagctgtagtgggaggctgcatcttccctaacctctgtctggcttgagcgttgacagagaaaaggcttagttctgaaaaccgatatgttgttggaagatgagcagccagatcactgcctaatctcgctttgctgtctgtgatgtagatggtggttcctatcctgagagcaagtgtgtttattcttttgcttctccccaataaagcacatgtttcatggtcaagccca

SEQ ID NO: 58 - DNA, 293 bp, synthetic construct
  source 1..293: mol_type = other DNA; note = Muscle_TUBB3
agctgctcgcagctggagtgagaggcaggtggcggccggggccgaagccagcagtgtctaaacccccggagccatcttgctgccgacaccctgctttcccctcgccctagggctcccttgccgccctcctgcagtatttatggcctcgtcctccccacctaggccacgtgtgagctgctcctgtctctgtcttattgcagctccaggcctgacgttttacggttttgttttttactggtttgtgtttatattttcggggatacttaataaatctattgctgtcagataccctt

SEQ ID NO: 59 - DNA, 234 bp, synthetic construct
  source 1..234: mol_type = other DNA; note = Spleen_CPN1
aacccacagtgccaggcaacccttcagaaaggctttgctcctgctctcagatcagatcaagcattctttctattttattatctgggacatatttaaatacaaacatattcagaacaattcagaatggtctccatctgttccaggggtaagccatctctaggtcatcatgaaaaaaattaggatctattgaaaggtgatgtggtggccgggtgtggtggctcacatctgtaatcc

SEQ ID NO: 60 - DNA, 164 bp, synthetic construct
  source 1..164: mol_type = other DNA; note = Spleen_LRRIQ1
aaatcacaaacgaattgatggaacctaatgccaacaagcattctttttcagatagggggtaggatgccagcaacctgaactgcccaaaaatgtgtatttaaattttttctttctttaaatatcctcttttgatataaacaaaattaaattatttctaaaattaa

SEQ ID NO: 61 - DNA, 112 bp, synthetic construct
  source 1..112: mol_type = other DNA; note = Spleen_MITD1
tgggtggtagcctaatttgtattatgtctactttaagtgaatattggattttttttaaaagatcacttttataatgtatgaatttaacaataaacttttatatttctactaa

SEQ ID NO: 62 - DNA, 296 bp, synthetic construct
  source 1..296: mol_type = other DNA; note = Spleen_RTN4R
cccccagcggacacaagagcgtgctcagcagccaggtgtgtgtacatacggggtctctctccacgccgccaagccagccgggcggccgacccgtggggcaggccaggccaggtcctccctgatggacgcctgccgcccgccacccccatctccaccccatcatgtttacagggttcggcggcagcgtttgttccagaacgccgcctcccacccagatcgcggtatatagagatatgcattttattttacttgtgtaaaaatatcggacgacgtggaataaagagctcttttcttaa

SEQ ID NO: 63 - DNA, 119 bp, synthetic construct
  source 1..119: mol_type = other DNA; note = Spleen_ZNF292
taattaatgtagtataaatacatcatttaccattttattttaaataggaagccatcaagcatgctagaattgtgaaactttcattatatttttttgttgttgacatgaattaacctggc

SEQ ID NO: 64 - DNA, 115 bp, synthetic construct
  source 1..115: mol_type = other DNA; note = Spleen_AIF1
tttgaagggaaaagggatgatgggattgaaggggcttctaatgacccagatatggaaacagaagacaaaattgtaagccagagtcaacaaattaaataaattaccccctcctcca

SEQ ID NO: 65 - DNA, 131 bp, synthetic construct
  source 1..131: mol_type = other DNA; note = Spleen_GZMM
tgccctggggtgatggggaccccctcgctgtctccacaggacccttcccctccaggggtgcagtggggtgggtgaggacgggtgggagggacagggagggaccaataaatcataatgaagaaacgctcaga

SEQ ID NO: 66 - DNA, 116 bp, synthetic construct
  source 1..116: mol_type = other DNA; note = Spleen_S100A12
gtagctctctgaaggctttttacccagcaatgtcctcaatgagggtcttttctttccctcaccaaaacccagccttgcccgtggggagtaagagttaataaacacactcacgaaaa

SEQ ID NO: 67 - DNA, 221 bp, synthetic construct
  source 1..221: mol_type = other DNA; note = Spleen_ALDH1L1
agaaaggtctttgtgagaagaaagtccctgcccctccctcgtggctggggccccctccctcttgagcctgggtgcacagcacctcccacctggggggctagtggaagccctcctgcctgcacaccatgtctgcatcttggacgccctctgtccagtcagaagcagcccttggctgggtgaggtgtgcccctcccagggagaataaagcttctgaagagaga

SEQ ID NO: 68 - DNA, 260 bp, synthetic construct
  source 1..260: mol_type = other DNA; note = Spleen_CRYM
aacaaaggaacttgatgttgagatggatgcttgaggaatattgctgctggttctcataatttctagagtaaatgagggagtccagtccccagtgaactctccttttgtgcttatcatgttttaccttaaatgctgagatcctcatttatgtttgtagttggaaagcaaagctaggtagccatttcttctgttctaccaagttataatagcattcatttccctttatatttccctgaaataaagcacattccaattgtgca

SEQ ID NO: 69 - DNA, 172 bp, synthetic construct
  source 1..172: mol_type = other DNA; note = Lymphoid_TTC6
ttacatagactgtggttgctatagtagtttacacagctgttctctctgaaacggaaacatatttgttgtctaaaaggttctaccattttcattattgtattcgttatgcttagtcttccatataaccttctatgcattttaataaaatgtttgttatacattaattataaaa

SEQ ID NO: 70 - DNA, 278 bp, synthetic construct
  source 1..278: mol_type = other DNA; note = Lymphoid_ZNF720
gagaccacccactaccacttcagaaaagcctggtgacctctctgcacactccatctgaagccatttatcacaacacagcccaggtgtgggaacagtaggcctattctctgctgacctgggagcagctgtctgagctcacctggctccaggggcctctgtgctgtggtacaaacctgtgccatggccacccaggtggcctatgtctttcgcactgagggctggctcatcccagccatactccctggtccctagggtggagaagctcagaactcctccta

SEQ ID NO: 71 - DNA, 322 bp, synthetic construct
  source 1..322: mol_type = other DNA; note = Lymphoid_ECM1
gtcaccccagagccctagagggtcagatggggggaaccccaccctgccccacccatctgaacactcattacactaaacacctcttggatttggtgtcctcattgtctatctaatgtctcacccgcagtgttttaagtggatcttggtgccctggcccaggagggcactggcgttttcagacacaccacagacaaacacaccctcctaagcctgcttgtatttccttcagtgcctggcccctgaggcccacggccctgcccccttcactgagcagatgttcacaggctgtgggatgcgaccataactaaacagcttgacgtca

SEQ ID NO: 72 - DNA, 296 bp, synthetic construct
  source 1..296: mol_type = other DNA; note = Lymphoid_RGS10
gcccccaaaaagccgggactggcagctttaagaagcaaaggaatttcctctcaggaccgtgccgggtttatcattgctttgttatttgtaaggactgaaatgtacaaaacccttcaatgggatgtgtgttttattaactgcttcaccagtaaattttgcatgatggctaagctaacataaaaaaagaataataataacttggaagttttagtttacaaaacagagattccttcaacactggacacgtcgagcattttgtagcttaattaaacctcatgtaaggccacaaggtgaaa

SEQ ID NO: 73 - DNA, 283 bp, synthetic construct
  source 1..283: mol_type = other DNA; note = Lymphoid_STMN1
gtacttaataaatatttgctgttgatgatagcaatgaccttgagactgatgaacagtctggccaagaggatccttgatgtggaagatagaaaaagcctttggggtcaggcagacttggattctaataccagccagttctgcttgctgtgtctgagcctcagtttactcatctgtgaagaggaggtagcaagaatgaaaatgcctgccttgtggtttgttgtaaggacagacactgccaacgtagagggcccagcagctcacagaccagttgctctgagagcag

SEQ ID NO: 74 - DNA, 174 bp, synthetic construct
  source 1..174: mol_type = other DNA; note = Lymphoid_CAMK2B
agagctgcgccctggtttcgccggacagagttggtgtttggagcccgactgccctcgggcacacggcctgcctgtcgcatgtttgtgtctgcctcgttccctcccctggtgcctgtgtctgcagaaaaacaagaccagatgtgatttgttaaaaaaaaacaaaaaaaaaaaaaa

SEQ ID NO: 75 - DNA, 284 bp, synthetic construct
  source 1..284: mol_type = other DNA; note = Lymphoid_EEF1A2
agcgcgggcgcccgcggcgcgaccctccccggcggtgccgcgctccgaaccccgggcccgggcccccgccccgcccccgccccgcgcgccggtccggcgccccgcacccccgccaggcgcatgtctgcacctccgcttgccagaggccctcggtcagcgactggatgctcgccatcaaggtccagtggaagttcttcaagaggaaaggcgcccccgccccaggcttccgcgcccagcgctcgccacgctcagtgcccgttttaccaataaactgagcgacccca

SEQ ID NO: 76 - DNA, 261 bp, synthetic construct
  source 1..261: mol_type = other DNA; note = Lymphoid_PYGM
gcctccagaccagaccccaaaccagcccttgagtctgtcacactctcttgggccagccccagcacctcatgcagagggtggggtactggagttagatctctaagcccctcctggaaccctcattttccccactctcaatgtcccagtgtccagcgtgactaaggacacgggcccccttccgtcctcgggctcccggtcccctcctatttatggggtctgaccaactgcacccactccctaataaattcattctccttggga

SEQ ID NO: 77 - DNA, 219 bp, synthetic construct
  source 1..219: mol_type = other DNA; note = Bone Marrow_FGD6
agatgagtaatttggggttttgtaatgccaactgcaagtaattacaatattttaaaaatccatttattttacataagattttttgctttgcttttggatgggggaggtgttgttgctgttatttttaatgtgaacagtgttcttgctttgtacctggagagctctttctcaaatgtgttaggaattttccatattattaaaatgcaatttttgtgtgtg

SEQ ID NO: 78 - DNA, 578 bp, synthetic construct
  source 1..578: mol_type = other DNA; note = Bone Marrow_KDM5D
cagtggcaccaaaggtcatttgtggttgtttttgtttgtttgtttcttaaatcctactatctcctggcctggacctcagaaggagctttttgcttatctataatttttcactgccaatttttgatatcctctctcctagagttactgttaaaaggttggttcgtaaagtccacaccccgatgctcagaagtgtcttgccagcaacattcctgctagcatacaggagtgatttcctaaaccagtttcattctagtctgaatagggacaaacaaatcttgaggaagcccaagtgcgtacctttatttttgcccccaccaccctctttctgtacttcaatttttgtttgttttttgtttttttgtccctgtcataaaatattttggtgcttcaaaacttgtaccttcattgtacatccttttcttttctccccttgggtcttattataaaagaagacaatgtacgttgtaattaccaaaaagaatagggaaaaacaagaatttcatgactctacctgtggtctatctttaatttcatttcttttgttaaaaataaaacaatgagtatgtttggatactatg

SEQ ID NO: 79 - DNA, 187 bp, synthetic construct
  source 1..187: mol_type = other DNA; note = Bone Marrow_RFX7
tggctagaactcaagcagccctcctggacttcatgttaaagacacatgctgaggatgattgagcaacaagatacaaggagcccagggcatgatgactttggaagggaagatgcccaactagtcctgactgcttacctctggatgtgttttacatgagagaaataaatgtctttctggtttaactcac

SEQ ID NO: 80 - DNA, 166 bp, synthetic construct
  source 1..166: mol_type = other DNA; note = Bone Marrow_RBM38
ccccgcactacatctacccaccagccatcgtgcagcccagcgtggtgatcccagccgcccctgtcccgtcgctgtcctcgccctacattgagtacacgccggccagcccggcctacgcccagtacccaccggccacctatgaccagtacccatacgccgcctcgcc

SEQ ID NO: 81 - DNA, 332 bp, synthetic construct
  source 1..332: mol_type = other DNA; note = Bone Marrow_SYNE3
cccactggggcacacaggtgactttctcctccaacctccatcagtcccagggcccctcctgaggatgctcgccagggaaactggaaacaggggcagggcaaagactgcagagctgcatccatatcagtgctgtgtcagcgttcccagaagacacttactttttatacagtgttgtcttagtctatttatactaaatgtgtactacatgtgactagggaataatgtctagaatttttatatgatctgtatgtaaatgctcagtatgtataatttcatatacgagttctatttggagttgggaaaattcctagcaatggctccctccaatggga

SEQ ID NO: 82 - DNA, 136 bp, synthetic construct
  source 1..136: mol_type = other DNA; note = Bone Marrow_VSTM1
caagaagacagccctggccactaaaggaggggggatcgtgctggccaaggttatcggaaatctggagatgcagatactgtgtttccttgctcttcgtccatatcaataaaattaagtttctcgtcttaaaaagaaa

SEQ ID NO: 83 - DNA, 136 bp, synthetic construct
  source 1..136: mol_type = other DNA; note = Bone Marrow_MT3
gaaggcacccctccgtgtggagcacgtggagatagtgccaggtggctcagtgccacctatgcctgtggtgaagtgtggctggtgtccccttcccctgctgaccttggaggaatgacaataaatcccatgaacagca

SEQ ID NO: 84 - DNA, 134 bp, synthetic construct
  source 1..134: mol_type = other DNA; note = Bone Marrow_VSNL1
gctgatgtcaatgctatggactgcacaaaagtctcaatgttccattcagtctgcagctattcacacacacacacacacacacacacacacacacacacacacacacaaatattgcttggactacctataaatgg

SEQ ID NO: 85 - DNA, 185 bp, synthetic construct
  source 1..185: mol_type = other DNA; note = High-RPKM_ACTB
gctgacctgggcaggtcggctgtggggtcctgtggtgtgtggggagctgtcacatccagggtcctcactgcctgtccccttccctcctcagatcattgctcctcctgagcgcaagtactccgtgtggatcggcggctccatcctggcctcgctgtccaccttccagcagatgtggatcagcaagc

SEQ ID NO: 86 - DNA, 295 bp, synthetic construct
  source 1..295: mol_type = other DNA; note = High-RPKM_EEF1A1
atattatccctaatacctgccaccccactcttaatcagtggtggaagaacggtctcagaactgtttgtttcaattggccatttaagtttagtagtaaaagactggttaatgataacaatgcatcgtaaaaccttcagaaggaaaggagaatgttttgtggaccactttggttttcttttttgcgtgtggcagttttaagttattagtttttaaaatcagtactttttaatggaaacaacttgaccaaaaatttgtcacagaattttgagacccattaaaaaagttaaatgagaaa

SEQ ID NO: 87 - DNA, 161 bp, synthetic construct
  source 1..161: mol_type = other DNA; note = High-RPKM_FTH1
gcctcgggctaatttccccatagccgtggggtgacttccctggtcaccaaggcagtgcatgcatgttggggtttcctttaccttttctataagttgtaccaaaacatccacttaagttctttgatttgtaccattccttcaaataaagaaatttggtaccc

SEQ ID NO: 88 - DNA, 144 bp, synthetic construct
  source 1..144: mol_type = other DNA
gagccttctgagcccagcgacttctgaagggccccttgcaaagtaatagggcttctgcctaagcctctccctccagccaataggcagctttcttaactatcctaacaagccttggaccaaatggaaataaagctttttgatgca

SEQ ID NO: 89 - DNA, 201 bp, synthetic construct
  source 1..201: mol_type = other DNA; note = High-RPKM_GAPDH
gacccctggaccaccagccccagcaagagcacaagaggaagagagagaccctcactgctggggagtccctgccacactcagtcccccaccacactgaatctcccctcctcacagttgccatgtagaccccttgaagaggggaggggcctagggagccgcaccttgtcatgtaccatcaataaagtaccctgtgctcaacca

SEQ ID NO: 90 - DNA, 293 bp, synthetic construct
  source 1..293: mol_type = other DNA; note = High-RPKM_HBB
tgttttctttccccttcttttctatggttaagttcatgtcataggaaggggataagtaacagggtacagtttagaatgggaaacagacgaatgattgcatcagtgtggaagtctcaggatcgttttagtttcttttatttgctgttcataacaattgttttcttttgtttaattcttgctttctttttttttcttctccgcaatttttactattatacttaatgccttaacattgtgtataacaaaaggaaatatctctgagatacattaagtaacttaaaaaaaaactttac

SEQ ID NO: 91 - DNA, 185 bp, synthetic construct
  source 1..185: mol_type = other DNA; note = High-RPKM_S100A9
gaccacagtggccaagatcacagtggccacggccacggccacagtcatggtggccacggccacagccactaatcaggaggccaggccaccctgcctctacccaaccagggccccggggcctgttatgtcaaactgtcttggctgtggggctaggggctggggccaaataaagtctcttcctccaa

SEQ ID NO: 92 - DNA, 270 bp, synthetic construct
  source 1..270: mol_type = other DNA; note = High-RPKM_TMSB4X
tgaggcgtgcgccgccaatatgcactgtacattccacaagcattgccttcttattttacttcttttagctgtttaactttgtaagatgcaaagaggttggatcaagtttaaatgactgtgctgcccctttcacatcaaagaactactgacaacgaaggccgcgcctgcctttcccatctgtctatctatctggctggcagggaaggaaagaacttgcatgttggtgaaggaagaagtggggtggaagaagtggggtgggacgacagtgaa

SEQ ID NO: 93 - DNA, 248 bp, synthetic construct
  source 1..248: mol_type = other DNA; note = High-RPKM_TMSB10
gatcctggaggatttcctacccccgtcctcttcgagaccccagtcgtgatgtggaggaagagccacctgcaagatggacacgagccacaagctgcactgtgaacctgggcactccgcgccgatgccaccggcctgtgggtctctgaagggacccccccccaatcggactgccaaattctccggtttgccccgggatattatagaaaattatttgtatgaataatgaaaataaaacacacctcgtggca

SEQ ID NO: 94 - DNA, 17 bp, synthetic construct
  source 1..17: mol_type = other DNA; note = promoter
taatacgactcactata

SEQ ID NO: 95 - skipped

SEQ ID NO: 96 - DNA, 840 bp, synthetic construct
  source 1..840: mol_type = other DNA; note = d2EGFP
gtgagcaagggcgaggagctgttcaccggggtggtgcccatcctggtcgagctggacggcgacgtaaacggccacaagttcagcgtgtccggcgagggcgagggcgatgccacctacggcaagctgaccctgaagttcatctgcaccaccggcaagctgcccgtgccctggcccaccctcgtgaccaccctgacctacggcgtgcagtgcttcagccgctaccccgaccacatgaagcagcacgacttcttcaagtccgccatgcccgaaggctacgtccaggagcgcaccatcttcttcaaggacgacggcaactacaagacccgcgccgaggtgaagttcgagggcgacaccctggtgaaccgcatcgagctgaagggcatcgacttcaaggaggacggcaacatcctggggcacaagctggagtacaactacaacagccacaacgtctatatcatggccgacaagcagaagaacggcatcaaggtgaacttcaagatccgccacaacatcgaggacggcagcgtgcagctcgccgaccactaccagcagaacacccccatcggcgacggccccgtgctgctgcccgacaaccactacctgagcacccagtccgccctgagcaaagaccccaacgagaagcgcgatcacatggtcctgctggagttcgtgaccgccgccgggatcactctcggcatggacgagctgtacaagaagcttagccatggcttcccgccggaggtggaggagcaggatgatggcacgctgcccatgtcttgtgcccaggagagcgggatggaccgtcaccctgcagcctgtgcttctgctaggatcaatgtg

SEQ ID NO: 97 - skipped

SEQ ID NO: 98 - DNA, 112 bp, synthetic construct
  source 1..112: mol_type = other DNA; note = poly A tail
aaaaaaaaaaaaaaaaaaaaaaaaaaaaaagcatatgactaaaaaaaaaaaaaaaaaaaaaaaaaaaaaaaaaaaaaaaaaaaaaaaaaaaaaaaaaaaaaaaaaaaaaaaa